European Patent Application EP 4 541 444 A1, published April 23, 2025. Title: Fusion protein for affinity capture. Applicant: Cytiva BioProcess R&D AB. Application EP. The sequence listing filed with the application follows.

SEQUENCE LISTING (235 sequences)

SEQ ID NO: 1 - protein, 58 aa, Staphylococcus aureus
ADNNFNKEQQNAFYEILNMPNLNEEQRNGFIQSLKDDPSQSANLLAEAKKLNESQAPK

SEQ ID NO: 2 - protein, 58 aa, Staphylococcus aureus [sequence omitted]

SEQ ID NO: 3 - protein, 58 aa, Staphylococcus aureus
ADNKFNKEQQNAFYEILHLPNLTEEQRNGFIQSLKDDPSVSKEILAEAKKLNDAQAPK

SEQ ID NO: 4 - protein, 61 aa, Staphylococcus aureus
ADAQQNKFNKDQQSAFYEILNMPNLNEEQRNGFIQSLKDDPSQSTNVLGEAKKLNESQAPK

SEQ ID NO: 5 - protein, 56 aa, Staphylococcus aureus
AQHDEAQQNAFYQVLNMPNLNADQRNGFIQSLKDDPSQSANVLGEAQKLNDSQAPK

SEQ ID NO: 6 - protein, 58 aa, synthetic construct [sequence omitted]

SEQ ID NO: 7 - protein, 58 aa, synthetic construct [sequence omitted]

SEQ ID NO: 8 - protein, 58 aa, synthetic construct
VDAKFDKEAQEAFYEILHLPNLTEEQRNAFIQSLKDDPSVSKAILAEAKKLNDAQAPK

SEQ ID NO: 9 - protein, 58 aa, synthetic construct
VDAKFDKEAQEAFYEILHLPNLTEEQRNAFIQSLKDDPSGSKAILAEAKKVNDAQAPK

SEQ ID NO: 10 - protein, 58 aa, synthetic construct
ADNNFNKEQQNAFYEILNMPNLNEEQRNGFIQALKDDPSRSANLLAEAKKINESQAPK

SEQ ID NO: 11 - protein, 58 aa, synthetic construct
ADNNFNKEQQNAFYEILNMPNLNEEQRNGFIQSLKDDPSGSANLLAEAKKVNESQAPK

SEQ ID NO: 12 - protein, 58 aa, synthetic construct
ADNNFNKEQQNAFYEILNMPNLNEEQRNGFIQALKDDPSGSANLLAEAKKRNESQAPK

SEQ ID NO: 13 - protein, 58 aa, synthetic construct
ADNKFNKEQQNAFYEILHLPNLNEEQRNGFIQALKDDPSRSANLLAEAKKINDAQAPK

SEQ ID NO: 14 - protein, 58 aa, synthetic construct
ADNKFNKEQQNAFYEILHLPNLNEEQRNGFIQSLKDDPSGSANLLAEAKKVNDAQAPK

SEQ ID NO: 15 - protein, 58 aa, synthetic construct
ADNKFNKEQQNAFYEILHLPNLNEEQRNGFIQALKDDPSGSANLLAEAKKRNDAQAPK

SEQ ID NO: 16 - protein, 58 aa, synthetic construct
ADNKFNKEQQNAFYEILHLPNLTEEQRNGFIQALKDDPSRSKEILAEAKKINDAQAPK

SEQ ID NO: 17 - protein, 58 aa, synthetic construct
ADNKFNKEQQNAFYEILHLPNLTEEQRNGFIQSLKDDPSGSKEILAEAKKVNDAQAPK

SEQ ID NO: 18 - protein, 58 aa, synthetic construct
ADNKFNKEQQNAFYEILHLPNLTEEQRNGFIQALKDDPSGSKEILAEAKKRNDAQAPK

SEQ ID NO: 19 - protein, 61 aa, synthetic construct
ADAQQNKFNKDQQSAFYEILNMPNLNEEQRNGFIQALKDDPSRSTNVLGEAKKINESQAPK

SEQ ID NO: 20 - protein, 61 aa, synthetic construct
ADAQQNKFNKDQQSAFYEILNMPNLNEEQRNGFIQSLKDDPSGSTNVLGEAKKVNESQAPK

SEQ ID NO: 21 - protein, 61 aa, synthetic construct
ADAQQNKFNKDQQSAFYEILNMPNLNEEQRNGFIQALKDDPSGSTNVLGEAKKRNESQAPK

SEQ ID NO: 22 - protein, 56 aa, synthetic construct
AQHDEAQQNAFYQVLNMPNLNADQRNGFIQALKDDPSRSANVLGEAQKINDSQAPK

SEQ ID NO: 23 - protein, 56 aa, synthetic construct
AQHDEAQQNAFYQVLNMPNLNADQRNGFIQALKDDPSGSANVLGEAQKRNDSQAPK

SEQ ID NO: 24 - protein, 56 aa, synthetic construct; identical to SEQ ID NO: 23

SEQ ID NO: 25 - protein, 58 aa, synthetic construct
VDNKFNKEQQNAFYEILHLPNLNEEQRNAFIQALKDDPSRSANLLAEAKKINDAQAPK

SEQ ID NO: 26 - protein, 58 aa, synthetic construct
VDNKFNKEQQNAFYEILHLPNLNEEQRNAFIQSLKDDPSGSANLLAEAKKVNDAQAPK

SEQ ID NO: 27 - protein, 58 aa, synthetic construct
VDNKFNKEQQNAFYEILHLPNLNEEQRNAFIQALKDDPSGSANLLAEAKKRNDAQAPK

SEQ ID NO: 28 - protein, 58 aa, synthetic construct
VDAKFDKEQQNAFYEILHLPNLTEEQRNAFIQALKDDPSRSANLLAEAKKINDAQAPK

SEQ ID NO: 29 - protein, 58 aa, synthetic construct
VDAKFDKEQQNAFYEILHLPNLTEEQRNAFIQSLKDDPSGSANLLAEAKKVNDAQAPK

SEQ ID NO: 30 - protein, 58 aa, synthetic construct
VDAKFDKEQQNAFYEILHLPNLTEEQRNAFIQALKDDPSGSANLLAEAKKRNDAQAPK

SEQ ID NO: 31 - protein, 58 aa, synthetic construct
ADNNFNKEAYRALAEIARMPNLNEEQRAGFIQSLKDDPSQSANLLAEAKKLNESQAPK

SEQ ID NO: 32 - protein, 58 aa, synthetic construct
ADNNFNKEAYRALAEIARMPNLNEESRAGFIQSLKDDPSQSANLLAEAKKLNESQAPK

SEQ ID NO: 33 - protein, 58 aa, synthetic construct
ADNKFNKEAYRALAEIARLPNLNEEQRAGFIQSLKDDPSQSANLLAEAKKLNDAQAPK

SEQ ID NO: 34 - protein, 58 aa, synthetic construct
ADNKFNKEAYRALAEIARLPNLNEESRAGFIQSLKDDPSQSANLLAEAKKLNDAQAPK

SEQ ID NO: 35 - protein, 58 aa, synthetic construct
ADNKFNKEAYEARAEIARLPNLNEEQRAGFIQSLKDDPSQSANLLAEAKKLNDAQAPK

SEQ ID NO: 36 - protein, 58 aa, synthetic construct
ADNKFNKEAYEARAEIALLPNLNEEQRAGFIQSLKDDPSQSANLLAEAKKLNDAQAPK

SEQ ID NO: 37 - protein, 58 aa, synthetic construct
ADNKFNKEAQRARAEILRLPNLNEEQRAGFIQSLKDDPSQSANLLAEAKKLNDAQAPK

SEQ ID NO: 38 - protein, 58 aa, synthetic construct
ADNKFNKEAYEALREIARLPNLNEEQRAGFIQSLKDDPSQSANLLAEAKKLNDAQAPK

SEQ ID NO: 39 - protein, 58 aa, synthetic construct
ADNKFNKEAYEAAREIARLPNLNEEQRAGFIQSLKDDPSQSANLLAEAKKLNDAQAPK

SEQ ID NO: 40 - protein, 58 aa, synthetic construct
ADNKFNKEYQRALAEIALLPNLNEEQRAGFIQSLKDDPSQSANLLAEAKKLNDAQAPK

SEQ ID NO: 41 - protein, 58 aa, synthetic construct
ADNKFNKEAYRALAEIARLPNLTEEQRAGFIQSLKDDPSVSKEILAEAKKLNDAQAPK

SEQ ID NO: 42 - protein, 58 aa, synthetic construct
ADNKFNKEAYRALAEIARLPNLTEESRAGFIQSLKDDPSVSKEILAEAKKLNDAQAPK

SEQ ID NO: 43 - protein, 58 aa, synthetic construct
ADNKFNKEAYEARAEIARLPNLTEEQRAGFIQSLKDDPSVSKEILAEAKKLNDAQAPK

SEQ ID NO: 44 - protein, 58 aa, synthetic construct
ADNKFNKEAYEARAEIALLPNLTEEQRAGFIQSLKDDPSVSKEILAEAKKLNDAQAPK

SEQ ID NO: 45 - protein, 58 aa, synthetic construct
ADNKFNKEAQRARAEILRLPNLTEEQRAGFIQSLKDDPSVSKEILAEAKKLNDAQAPK

SEQ ID NO: 46 - protein, 58 aa, synthetic construct
ADNKFNKEAYEALREIARLPNLTEEQRAGFIQSLKDDPSVSKEILAEAKKLNDAQAPK

SEQ ID NO: 47 - protein, 58 aa, synthetic construct
ADNKFNKEAYEAAREIARLPNLTEEQRAGFIQSLKDDPSVSKEILAEAKKLNDAQAPK

SEQ ID NO: 48 - protein, 58 aa, synthetic construct
ADNKFNKEYQRALAEIALLPNLTEEQRAGFIQSLKDDPSVSKEILAEAKKLNDAQAPK

SEQ ID NO: 49 - protein, 61 aa, synthetic construct
ADAQQNKFNKDAYRALAEIARMPNLNEEQRAGFIQSLKDDPSQSTNVLGEAKKLNESQAPK

SEQ ID NO: 50 - protein, 61 aa, synthetic construct
ADAQQNKFNKDAYRALAEIARMPNLNEESRAGFIQSLKDDPSQSTNVLGEAKKLNESQAPK

SEQ ID NO: 51 - protein, 56 aa, synthetic construct
AQHDEAAYRALAQVARMPNLNADQRAGFIQSLKDDPSQSANVLGEAQKLNDSQAPK

SEQ ID NO: 52 - protein, 56 aa, synthetic construct
AQHDEAAYRALAQVARMPNLNADSRAGFIQSLKDDPSQSANVLGEAQKLNDSQAPK

SEQ ID NO: 53 - protein, 56 aa, synthetic construct
AQHDEAAYEARAQVARMPNLNADQRAGFIQSLKDDPSQSANVLGEAQKLNDSQAPK

SEQ ID NO: 54 - protein, 56 aa, synthetic construct
AQHDEAAYEARAQVALMPNLNADQRAGFIQSLKDDPSQSANVLGEAQKLNDSQAPK

SEQ ID NO: 55 - protein, 56 aa, synthetic construct
AQHDEAAQRARAQVLRMPNLNADQRAGFIQSLKDDPSQSANVLGEAQKLNDSQAPK

SEQ ID NO: 56 - protein, 56 aa, synthetic construct
AQHDEAAYEALRQVARMPNLNADQRAGFIQSLKDDPSQSANVLGEAQKLNDSQAPK

SEQ ID NO: 57 - protein, 56 aa, synthetic construct
AQHDEAAYEAARQVARMPNLNADQRAGFIQSLKDDPSQSANVLGEAQKLNDSQAPK

SEQ ID NO: 58 - protein, 56 aa, synthetic construct
AQHDEAYQRALAQVALMPNLNADQRAGFIQSLKDDPSQSANVLGEAQKLNDSQAPK

SEQ ID NO: 59 - protein, 58 aa, synthetic construct
VDNKFNKEAYRALAEIARLPNLNEEQRAGFIQSLKDDPSQSANLLAEAKKLNDAQAPK

SEQ ID NO: 60 - protein, 58 aa, synthetic construct
VDNKFNKEAYRALAEIARLPNLNEESRAGFIQSLKDDPSQSANLLAEAKKLNDAQAPK

SEQ ID NO: 61 - protein, 58 aa, synthetic construct
VDAKFDKEAYRALAEIARLPNLTEEQRAGFIQSLKDDPSQSANLLAEAKKLNDAQAPK

SEQ ID NO: 62 - protein, 58 aa, synthetic construct
VDAKFDKEAYRALAEIARLPNLTEESRAGFIQSLKDDPSQSANLLAEAKKLNDAQAPK

SEQ ID NO: 63 - protein, 58 aa, synthetic construct
VDAKFDKEAYRALAEIARLPNLTEEQRAGFIQSLKDDPSVSKAILAEAKKLNDAQAPK

SEQ ID NO: 64 - protein, 58 aa, synthetic construct
VDAKFDKEAYRALAEIARLPNLTEEQRAAFIQSLKDDPSGSKAILAEAKKVNDAQAPK

SEQ ID NO: 65 - protein, 58 aa, synthetic construct
VDAKFDKEAYRALAEIARLPNLTEEQRLAFIQSLKDDPSGSKAILAEAKKVNDAQAPK

SEQ ID NO: 66 - protein, 58 aa, synthetic construct
VDAKFDKEAYRALAEIARLPNLTEEQREAFIQSLKDDPSGSKAILAEAKKVNDAQAPK

SEQ ID NO: 67 - protein, 58 aa, synthetic construct
VDAKFDKEAYRALAEIARLPNLTEEQRRAFIQSLKDDPSGSKAILAEAKKVNDAQAPK

SEQ ID NO: 68 - protein, 58 aa, synthetic construct
VDAKFDKEAYRALAEIARLPNLTEEQRALFIQSLKDDPSGSKAILAEAKKVNDAQAPK

SEQ ID NO: 69 - protein, 58 aa, synthetic construct
VDAKFDKEAYRALAEIARLPNLTEEQRAEFIQSLKDDPSGSKAILAEAKKVNDAQAPK

SEQ ID NO: 70 - protein, 58 aa, synthetic construct
VDAKFDKEAYRALAEIARLPNLTEEQRARFIQSLKDDPSGSKAILAEAKKVNDAQAPK

SEQ ID NO: 71 - protein, 58 aa, synthetic construct
VDAKFDKEAYRALAEIARLPNLTEEQRAAFIQTLKDDPSESKAILAEAKKRNDAQAPK

SEQ ID NO: 72 - protein, 58 aa, synthetic construct
VDAKFDKEAYRALAEIARLPNLTEEQRAAFIQALKDDPSRSKAILAEAKKINDAQAPK

SEQ ID NO: 73 - protein, 58 aa, synthetic construct
VDAKFDKEAYRALAEIARLPNLTEEQRAAFIQALKDDPSGSKAILAEAKKRNDAQAPK

SEQ ID NO: 74 - protein, 58 aa, synthetic construct
VDAKFDKEAYRALAEIARLPNLTEEQRAAFIQQLKDDPSDSKAILAEAKKINDAQAPK

SEQ ID NO: 75 - protein, 58 aa, synthetic construct
VDAKFDKEAYRALAEIARLPNLTEEQRAAFIQGLKDDPSRSKAILAEAKKLNDAQAPK

SEQ ID NO: 76 - protein, 58 aa, synthetic construct
VDAKFDKEAYRALAEIARLPNLTEEQRAAFIQHLKDDPSKSKAILAEAKKLNDAQAPK

SEQ ID NO: 77 - protein, 58 aa, synthetic construct
VDAKFDKEAYRALAEIARLPNLTEEQRAAFIQELKDDPSGSKAILAEAKKLNDAQAPK

SEQ ID NO: 78 - protein, 58 aa, synthetic construct
VDAKFDKERYRALAEIARLPNLTEEQRAAFIQSLKDDPSGSKAILAEAKKVNDAQAPK

SEQ ID NO: 79 - protein, 58 aa, synthetic construct
VDAKFDKEAYRALAEILRLPNLTEEQRAAFIQSLKDDPSGSKAILAEAKKVNDAQAPK

SEQ ID NO: 80 - protein, 58 aa, synthetic construct
VDAKFDKEAYRALAEIAELPNLTEEQRAAFIQSLKDDPSGSKAILAEAKKVNDAQAPK

SEQ ID NO: 81 - protein, 58 aa, synthetic construct
VDAKFDKEAYRALAEIALLPNLTEEQRAAFIQSLKDDPSGSKAILAEAKKVNDAQAPK

SEQ ID NO: 82 - protein, 58 aa, synthetic construct
VDAKFDKEAYRALAEIELLPNLTEEQRAAFIQSLKDDPSGSKAILAEAKKVNDAQAPK

SEQ ID NO: 83 - protein, 58 aa, synthetic construct
VDAKFDKEAYRALAEIEALPNLTEEQRAAFIQSLKDDPSGSKAILAEAKKVNDAQAPK

SEQ ID NO: 84 - protein, 58 aa, synthetic construct
VDAKFDKEAYRALAEILALPNLTEEQRAAFIQSLKDDPSGSKAILAEAKKVNDAQAPK

SEQ ID NO: 85 - protein, 58 aa, synthetic construct
VDAKFDKEAYRALAEILELPNLTEEQRAAFIQSLKDDPSGSKAILAEAKKVNDAQAPK

SEQ ID NO: 86 - protein, 58 aa, synthetic construct
VDAKFDKEAYRALAEIRALPNLTEEQRAAFIQSLKDDPSGSKAILAEAKKVNDAQAPK

SEQ ID NO: 87 - protein, 58 aa, synthetic construct
VDAKFDKEAYRALAEIRELPNLTEEQRAAFIQSLKDDPSGSKAILAEAKKVNDAQAPK

SEQ ID NO: 88 - protein, 58 aa, synthetic construct
VDAKFDKEAYRALAEIRLLPNLTEEQRAAFIQSLKDDPSGSKAILAEAKKVNDAQAPK

SEQ ID NO: 89 - protein, 58 aa, synthetic construct
VDAKFDKEAYRALAEIRRLPNLTEEQRAAFIQSLKDDPSGSKAILAEAKKVNDAQAPK

SEQ ID NO: 90 - protein, 58 aa, synthetic construct
VDAKFDKEAYRALQEIARLPNLTEEQRAAFIQSLKDDPSGSKAILAEAKKVNDAQAPK

SEQ ID NO: 91 - protein, 58 aa, synthetic construct
VDAKFDKEAYRAELEIARLPNLTEEQRAAFIQSLKDDPSGSKAILAEAKKVNDAQAPK

SEQ ID NO: 92 - protein, 58 aa, synthetic construct
VDAKFDKEAYRARAEIARLPNLTEEQRAAFIQSLKDDPSGSKAILAEAKKVNDAQAPK

SEQ ID NO: 93 - protein, 58 aa, synthetic construct
VDAKFDKEAYRAAREIARLPNLTEEQRAAFIQSLKDDPSGSKAILAEAKKVNDAQAPK

SEQ ID NO: 94 - protein, 58 aa, synthetic construct
VDAKFDKEAYRAQAEIARLPNLTEEQRAAFIQSLKDDPSGSKAILAEAKKVNDAQAPK

SEQ ID NO: 95 - protein, 58 aa, synthetic construct
VDAKFDKEAYRALEEIARLPNLTEEQRAAFIQSLKDDPSGSKAILAEAKKVNDAQAPK

SEQ ID NO: 96 - protein, 58 aa, synthetic construct
VDAKFDKEAYRAEREIARLPNLTEEQRAAFIQSLKDDPSGSKAILAEAKKVNDAQAPK

SEQ ID NO: 97 - protein, 58 aa, synthetic construct
VDAKFDKEAYRARLEIARLPNLTEEQRAAFIQSLKDDPSGSKAILAEAKKVNDAQAPK

SEQ ID NO: 98 - protein, 58 aa, synthetic construct
VDAKFDKEAYRAAQEIARLPNLTEEQRAAFIQSLKDDPSGSKAILAEAKKVNDAQAPK

SEQ ID NO: 99 - protein, 58 aa, synthetic construct
VDAKFDKEAYRAQEEIARLPNLTEEQRAAFIQSLKDDPSGSKAILAEAKKVNDAQAPK

SEQ ID NO: 100 - protein, 58 aa, synthetic construct
VDAKFDKEAYRAQQEIARLPNLTEEQRAAFIQSLKDDPSGSKAILAEAKKVNDAQAPK

SEQ ID NO: 101 - protein, 58 aa, synthetic construct
VDAKFDKEAYRARREIARLPNLTEEQRAAFIQSLKDDPSGSKAILAEAKKVNDAQAPK

SEQ ID NO: 102 - protein, 58 aa, synthetic construct
VDAKFDKERYRAAREIERLPNLTEEQREAFIQSLKDDPSGSKAILAEAKKRNDAQAPK

SEQ ID NO: 103 - protein, 58 aa, synthetic construct
VDAKFDKEERLAQAEIAALPNLTEEQRALFIQALKDDPSRSKAILAEAKKINDAQAPK

SEQ ID NO: 104 - protein, 58 aa, synthetic construct
VDAKFDKEYAEARLEIRALPNLTEEQRARFIQALKDDPSGSKAILAEAKKVNDAQAPK

SEQ ID NO: 105 - protein, 58 aa, synthetic construct
VDAKFDKEERAAEREIARLPNLTEEQRRRFIQSLKDDPSGSKAILAEAKKVNDAQAPK

SEQ ID NO: 106 - protein, 58 aa, synthetic construct
VDAKFDKERALARREIELLPNLTEEQRAAFIQALKDDPSGSKAILAEAKKRNDAQAPK

SEQ ID NO: 107 - protein, 58 aa, synthetic construct
VDAKFDKELYRALAEIARLPNLTEEQRALFIQSLKDDPSGSKAILAEAKKSNDAQAPK

SEQ ID NO: 108 - protein, 58 aa, synthetic construct
VDAKFDKEAYLALAEIARLPNLTEEQRALFIQSLKDDPSSSKAILAEAKKGNDAQAPK

SEQ ID NO: 109 - protein, 58 aa, synthetic construct
VDAKFDKEAYRALAEIARLPNLTEEQRAAFIQRLKDDPSHSKAILAEAKKVNDAQAPK

SEQ ID NO: 110 - protein, 58 aa, synthetic construct
VDAKFDKEAYAAKAEIARLPNLTEEQRAAFIQSLKDDPSQSKAILAEAKKVNDAQAPK

SEQ ID NO: 111 - protein, 128 aa, synthetic construct
VDQLQESGGGSVQAGEALRLSCVGSGYTSINPYMAWFRQAPGKEREGVAAISSGGVYTYYADSVKGRFTITRDNVKNTMYLQMPSLKPEDSAKYYCAADFRRGGNWNVDPFRYDYQHWGQGTQVTVSS

SEQ ID NO: 112 - protein, 197 aa, synthetic construct
VDQLQESGGGSVQAGEALRLSCVGSGYTSINPYMAWFRQAPGKEREGVAAISSGGVYTYYADSVKGRFTITRDNVKNTMYLQMPSLKPEDSAKYYCAADFRRGGNWNVDPFRYDYQHWGQGTQVTVSSQASVDAKFDKEAYRALAEIARLPNLTEEQRAAFIQSLKDDPSGSKAILAEAKKVNDAQAPKGSHHHHHH

SEQ ID NO: 113 - protein, 128 aa, synthetic construct
QVQLQESGGGLVQPGGSLRLSCAASGRTSINPYMAWFRQAPGKQREFVAAISSGGVYTYYTDSVKGRFTISRDNAKTTVYLQMNSLKPEDTAVYYCAADFRRGGNWNVDPFRYDYQYWGQGTQVTVSS

SEQ ID NO: 114 - protein, 137 aa, synthetic construct
QVQLQESGGGLVQPGGSLRLSCAASGRTSINPYMAWFRQAPGKQREFVAAISSGGVYTYYTDSVKGRFTISRDNAKTTVYLQMNSLKPEDTAVYYCAADFRRGGNWNVDPFRYDYQYWGQGTQVTVSSQASHHHHHH

SEQ ID NO: 115 - protein, 202 aa, synthetic construct
  SIGNAL 1..4
AQGTQVQLQESGGGLVQPGGSLRLSCAASGRTSINPYMAWFRQAPGKQREFVAAISSGGVYTYYTDSVKGRFTISRDNAKTTVYLQMNSLKPEDTAVYYCAADFRRGGNWNVDPFRYDYQYWGQGTQVTVSSQASVDAKFDKEAQEAFYEILHLPNLTEEQRNAFIQSLKDDPSGSKAILAEAKKVNDAQAPKGSHHHHHHC

SEQ ID NO: 116 - protein, 197 aa, synthetic construct
QVQLQESGGGLVQPGGSLRLSCAASGRTSINPYMAWFRQAPGKQREFVAAISSGGVYTYYTDSVKGRFTISRDNAKTTVYLQMNSLKPEDTAVYYCAADFRRGGNWNVDPFRYDYQYWGQGTQVTVSSQASVDAKFDKEAYRALAEIARLPNLTEEQRAAFIQSLKDDPSGSKAILAEAKKVNDAQAPKGSHHHHHH

SEQ ID NO: 117 - protein, 197 aa, synthetic construct
QVQLQESGGGLVQPGGSLRLSCAASGRTSINPYMAWFRQAPGKQREFVAAISSGGVYTYYTDSVKGRFTISRDNAKTTVYLQMNSLKPEDTAVYYCAADFRRGGNWNVDPFRYDYQYWGQGTQVTVSSQASADNKFNKEQQNAFYEILHLPNLNEEQRNGFIQSLKDDPSGSANLLAEAKKVNDAQAPKGSHHHHHH

SEQ ID NO: 118 - protein, 197 aa, synthetic construct
QVQLQESGGGLVQPGGSLRLSCAASGRTSINPYMAWFRQAPGKQREFVAAISSGGVYTYYTDSVKGRFTISRDNAKTTVYLQMNSLKPEDTAVYYCAADFRRGGNWNVDPFRYDYQYWGQGTQVTVSSQASVDNKFNKEQQNAFYEILHLPNLNEEQRNAFIQSLKDDPSGSANLLAEAKKVNDAQAPKGSHHHHHH

SEQ ID NO: 119 - protein, 197 aa, synthetic construct
QVQLQESGGGLVQPGGSLRLSCAASGRTSINPYMAWFRQAPGKQREFVAAISSGGVYTYYTDSVKGRFTISRDNAKTTVYLQMNSLKPEDTAVYYCAADFRRGGNWNVDPFRYDYQYWGQGTQVTVSSQASVDAKFDKEQQNAFYEILHLPNLTEEQRNAFIQSLKDDPSGSANLLAEAKKVNDAQAPKGSHHHHHH

SEQ ID NO: 120 - protein, 128 aa, synthetic construct
QVQLQQSGGGSVQAGGSLRLSCTISGRTSINPYMAWFRQRPGKEREFVAAISSGGVYTYYADSVKGRFTISRDNAKNTVYLQMNSLKPEDTAVYYCAADFRRGGNWNVDPFRYDYDYWGQGTQVTVSS

SEQ ID NO: 121 - protein, 137 aa, synthetic construct
QVQLQQSGGGSVQAGGSLRLSCTISGRTSINPYMAWFRQRPGKEREFVAAISSGGVYTYYADSVKGRFTISRDNAKNTVYLQMNSLKPEDTAVYYCAADFRRGGNWNVDPFRYDYDYWGQGTQVTVSSQASHHHHHH

SEQ ID NO: 122 - protein, 202 aa, synthetic construct
  SIGNAL 1..4
AQGTQVQLQQSGGGSVQAGGSLRLSCTISGRTSINPYMAWFRQRPGKEREFVAAISSGGVYTYYADSVKGRFTISRDNAKNTVYLQMNSLKPEDTAVYYCAADFRRGGNWNVDPFRYDYDYWGQGTQVTVSSQASVDAKFDKEAQEAFYEILHLPNLTEEQRNAFIQSLKDDPSGSKAILAEAKKVNDAQAPKGSHHHHHHC

SEQ ID NO: 123 - protein, 197 aa, synthetic construct
QVQLQQSGGGSVQAGGSLRLSCTISGRTSINPYMAWFRQRPGKEREFVAAISSGGVYTYYADSVKGRFTISRDNAKNTVYLQMNSLKPEDTAVYYCAADFRRGGNWNVDPFRYDYDYWGQGTQVTVSSQASVDAKFDKEAYRALAEIARLPNLTEEQRAAFIQSLKDDPSGSKAILAEAKKVNDAQAPKGSHHHHHH

SEQ ID NO: 124 - protein, 197 aa, synthetic construct
QVQLQQSGGGSVQAGGSLRLSCTISGRTSINPYMAWFRQRPGKEREFVAAISSGGVYTYYADSVKGRFTISRDNAKNTVYLQMNSLKPEDTAVYYCAADFRRGGNWNVDPFRYDYDYWGQGTQVTVSSQASADNKFNKEQQNAFYEILHLPNLNEEQRNGFIQSLKDDPSGSANLLAEAKKVNDAQAPKGSHHHHHH

SEQ ID NO: 125 - protein, 197 aa, synthetic construct
QVQLQQSGGGSVQAGGSLRLSCTISGRTSINPYMAWFRQRPGKEREFVAAISSGGVYTYYADSVKGRFTISRDNAKNTVYLQMNSLKPEDTAVYYCAADFRRGGNWNVDPFRYDYDYWGQGTQVTVSSQASVDNKFNKEQQNAFYEILHLPNLNEEQRNAFIQSLKDDPSGSANLLAEAKKVNDAQAPKGSHHHHHH

SEQ ID NO: 126 - protein, 197 aa, synthetic construct
QVQLQQSGGGSVQAGGSLRLSCTISGRTSINPYMAWFRQRPGKEREFVAAISSGGVYTYYADSVKGRFTISRDNAKNTVYLQMNSLKPEDTAVYYCAADFRRGGNWNVDPFRYDYDYWGQGTQVTVSSQASVDAKFDKEQQNAFYEILHLPNLTEEQRNAFIQSLKDDPSGSANLLAEAKKVNDAQAPKGSHHHHHH

SEQ ID NO: 127 - protein, 127 aa, Lama glama
EVQLVESGGGLVQAGGSLRLSCAASGRTFSSYAMGWFRQAPGKEREFVVAINWSSGSTYYADSVKGRFTISRDNAKNTMYLQMNSLKPEDTAVYYCAAGYQINSGNYNFKDYEYDYWGQGTQVTVSS

SEQ ID NO: 128 - protein, 127 aa, synthetic construct
QVQLQQSGGGSVQAGGSLRLSCTISGRTFSSYAMGWFRQRPGKEREFVAAINWSSGSTYYADSVKGRFTISRDNAKNTVYLQMNSLKPEDTAVYYCAAGYQINSGNYNFKDYEYDYWGQGTQVTVSS

SEQ ID NO: 129 - protein, 197 aa, synthetic construct
EVQLVESGGGLVQAGGSLRLSCAASGRTFSSYAMGWFRQAPGKEREFVVAINWSSGSTYYADSVKGRFTISRDNAKNTMYLQMNSLKPEDTAVYYCAAGYQINSGNYNFKDYEYDYWGQGTQVTVSSQASVDAKFDKEAQEAFYEILHLPNLTEEQRNAFIQSLKDDPSGSKAILAEAKKVNDAQAPKGSHHHHHHC

SEQ ID NO: 130 - protein, 197 aa, synthetic construct
QVQLQQSGGGSVQAGGSLRLSCTISGRTFSSYAMGWFRQRPGKEREFVAAINWSSGSTYYADSVKGRFTISRDNAKNTVYLQMNSLKPEDTAVYYCAAGYQINSGNYNFKDYEYDYWGQGTQVTVSSQASVDAKFDKEAQEAFYEILHLPNLTEEQRNAFIQSLKDDPSGSKAILAEAKKVNDAQAPKGSHHHHHHC

SEQ ID NO: 131 - protein, 196 aa, synthetic construct
EVQLVESGGGLVQAGGSLRLSCAASGRTFSSYAMGWFRQAPGKEREFVVAINWSSGSTYYADSVKGRFTISRDNAKNTMYLQMNSLKPEDTAVYYCAAGYQINSGNYNFKDYEYDYWGQGTQVTVSSQASVDAKFDKEAYRALAEIARLPNLTEEQRAAFIQSLKDDPSGSKAILAEAKKVNDAQAPKGSHHHHHH

SEQ ID NO: 132 - protein, 196 aa, synthetic construct
QVQLQQSGGGSVQAGGSLRLSCTISGRTFSSYAMGWFRQRPGKEREFVAAINWSSGSTYYADSVKGRFTISRDNAKNTVYLQMNSLKPEDTAVYYCAAGYQINSGNYNFKDYEYDYWGQGTQVTVSSQASVDAKFDKEAYRALAEIARLPNLTEEQRAAFIQSLKDDPSGSKAILAEAKKVNDAQAPKGSHHHHHH

SEQ ID NO: 133 - protein, 126 aa, synthetic construct
QVQLQESGGGLVQPGGSLRLSCAASGRTLSDYTMGWFRQAPGKQREFVAAISWSGAYTKYTDSVKGRFTISRDNAKTTVYLQMNSLKPEDTAVYYCAAGPTGLLSKKATPADYDYWGQGTQVTVSS

SEQ ID NO: 134 - protein, 195 aa, synthetic construct
QVQLQESGGGLVQPGGSLRLSCAASGRTLSDYTMGWFRQAPGKQREFVAAISWSGAYTKYTDSVKGRFTISRDNAKTTVYLQMNSLKPEDTAVYYCAAGPTGLLSKKATPADYDYWGQGTQVTVSSQASVDAKFDKEAYRALAEIARLPNLTEEQRAAFIQSLKDDPSGSKAILAEAKKVNDAQAPKGSHHHHHH

SEQ ID NO: 135 - protein, 126 aa, synthetic construct
EVQLVESGGGLVQAGGSLRLSCAASGRTLSDYTMGWFRQAPGKEREFVVAISWSGAYTKYADSVKGRFTISRDNAKNTMYLQMNSLKPEDTAVYYCAAGPTGLLSKKATPADYDYWGQGTQVTVSS

SEQ ID NO: 136 - protein, 195 aa, synthetic construct
EVQLVESGGGLVQAGGSLRLSCAASGRTLSDYTMGWFRQAPGKEREFVVAISWSGAYTKYADSVKGRFTISRDNAKNTMYLQMNSLKPEDTAVYYCAAGPTGLLSKKATPADYDYWGQGTQVTVSSQASVDAKFDKEAYRALAEIARLPNLTEEQRAAFIQSLKDDPSGSKAILAEAKKVNDAQAPKGSHHHHHH

SEQ ID NO: 137 - protein, 126 aa, synthetic construct
QVQLQESGGGSVQAGGSLRLSCVASGRTLSDYTMGWFRQPPGKAREFVAAISWSGAYTKYADSVKGRFTISRDNAKNTVYLQMNSLKPEDTAVYYCAAGPTGLLSKKATPADYDYWGQGTQVTVSS

SEQ ID NO: 138 - protein, 200 aa, synthetic construct
  SIGNAL 1..4
AQGTQVQLQESGGGSVQAGGSLRLSCVASGRTLSDYTMGWFRQPPGKAREFVAAISWSGAYTKYADSVKGRFTISRDNAKNTVYLQMNSLKPEDTAVYYCAAGPTGLLSKKATPADYDYWGQGTQVTVSSQASVDAKFDKEAQEAFYEILHLPNLTEEQRNAFIQSLKDDPSGSKAILAEAKKVNDAQAPKGSHHHHHHC

SEQ ID NO: 139 - protein, 126 aa, synthetic construct
QVQLQQSGGGSVQAGGSLRLSCTISGRTLSDYTMGWFRQRPGKEREFVAAISWSGAYTKYADSVKGRFTISRDNAKNTVYLQMNSLKPEDTAVYYCAAGPTGLLSKKATPADYDYWGQGTQVTVSS

SEQ ID NO: 140 - protein, 135 aa, synthetic construct
QVQLQQSGGGSVQAGGSLRLSCTISGRTLSDYTMGWFRQRPGKEREFVAAISWSGAYTKYADSVKGRFTISRDNAKNTVYLQMNSLKPEDTAVYYCAAGPTGLLSKKATPADYDYWGQGTQVTVSSQASHHHHHH

SEQ ID NO: 141 - protein, 200 aa, synthetic construct
  SIGNAL 1..4
AQGTQVQLQQSGGGSVQAGGSLRLSCTISGRTLSDYTMGWFRQRPGKEREFVAAISWSGAYTKYADSVKGRFTISRDNAKNTVYLQMNSLKPEDTAVYYCAAGPTGLLSKKATPADYDYWGQGTQVTVSSQASVDAKFDKEAQEAFYEILHLPNLTEEQRNAFIQSLKDDPSGSKAILAEAKKVNDAQAPKGSHHHHHHC

SEQ ID NO: 142 - protein, 195 aa, synthetic construct
QVQLQQSGGGSVQAGGSLRLSCTISGRTLSDYTMGWFRQRPGKEREFVAAISWSGAYTKYADSVKGRFTISRDNAKNTVYLQMNSLKPEDTAVYYCAAGPTGLLSKKATPADYDYWGQGTQVTVSSQASVDAKFDKEAYRALAEIARLPNLTEEQRAAFIQSLKDDPSGSKAILAEAKKVNDAQAPKGSHHHHHH

SEQ ID NO: 143 - protein, 420 aa, synthetic construct
QVQLQQSGGGSVQAGGSLRLSCTISGRTLSDYTMGWFRQRPGKEREFVAAISWSGAYTKYADSVKGRFTISRDNAKNTVYLQMNSLKPEDTAVYYCAAGPTGLLSKKATPADYDYWGQGTQVTVSSQASAEAAAKEAAAKAGQVQLQQSGGGSVQAGGSLRLSCTISGRTLSDYTMGWFRQRPGKEREFVAAISWSGAYTKYADSVKGRFTISRDNAKNTVYLQMNSLKPEDTAVYYCAAGPTGLLSKKATPADYDYWGQGTQVTVSSQASAEAAAKEAAAKAGQVQLQQSGGGSVQAGGSLRLSCTISGRTLSDYTMGWFRQRPGKEREFVAAISWSGAYTKYADSVKGRFTISRDNAKNTVYLQMNSLKPEDTAVYYCAAGPTGLLSKKATPADYDYWGQGTQVTVSSQASHHHHHHC

SEQ ID NO: 144 - protein, 480 aa, synthetic construct
QVQLQQSGGGSVQAGGSLRLSCTISGRTLSDYTMGWFRQRPGKEREFVAAISWSGAYTKYADSVKGRFTISRDNAKNTVYLQMNSLKPEDTAVYYCAAGPTGLLSKKATPADYDYWGQGTQVTVSSQASAEAAAKEAAAKAGQVQLQQSGGGSVQAGGSLRLSCTISGRTLSDYTMGWFRQRPGKEREFVAAISWSGAYTKYADSVKGRFTISRDNAKNTVYLQMNSLKPEDTAVYYCAAGPTGLLSKKATPADYDYWGQGTQVTVSSQASAEAAAKEAAAKAGQVQLQQSGGGSVQAGGSLRLSCTISGRTLSDYTMGWFRQRPGKEREFVAAISWSGAYTKYADSVKGRFTISRDNAKNTVYLQMNSLKPEDTAVYYCAAGPTGLLSKKATPADYDYWGQGTQVTVSSQASVDAKFDKEAYRALAEIARLPNLTEEQRAAFIQSLKDDPSGSKAILAEAKKVNDAQAPKGSHHHHHHC

SEQ ID NO: 145 - protein, 596 aa, synthetic construct
QVQLQQSGGGSVQAGGSLRLSCTISGRTLSDYTMGWFRQRPGKEREFVAAISWSGAYTKYADSVKGRFTISRDNAKNTVYLQMNSLKPEDTAVYYCAAGPTGLLSKKATPADYDYWGQGTQVTVSSQASVDAKFDKEAYRALAEIARLPNLTEEQRAAFIQSLKDDPSGSKAILAEAKKVNDAQAPKAEAAAKEAAAKAGQVQLQQSGGGSVQAGGSLRLSCTISGRTLSDYTMGWFRQRPGKEREFVAAISWSGAYTKYADSVKGRFTISRDNAKNTVYLQMNSLKPEDTAVYYCAAGPTGLLSKKATPADYDYWGQGTQVTVSSQASVDAKFDKEAYRALAEIARLPNLTEEQRAAFIQSLKDDPSGSKAILAEAKKVNDAQAPKAEAAAKEAAAKAGQVQLQQSGGGSVQAGGSLRLSCTISGRTLSDYTMGWFRQRPGKEREFVAAISWSGAYTKYADSVKGRFTISRDNAKNTVYLQMNSLKPEDTAVYYCAAGPTGLLSKKATPADYDYWGQGTQVTVSSQASVDAKFDKEAYRALAEIARLPNLTEEQRAAFIQSLKDDPSGSKAILAEAKKVNDAQAPKGSHHHHHHC

SEQ ID NO: 146 - protein, 83 aa, synthetic construct
VDPKEEVTIKANLIYADGKTQTAEFKGTFEEATAEAYRYADLLAKENGKYTVDVADKGYTLNIKFAGKEKTPEEKASHHHHHH

SEQ ID NO: 147 - protein, 143 aa, synthetic construct
VDPKEEVTIKANLIYADGKTQTAEFKGTFEEATAEAYRYADLLAKENGKYTVDVADKGYTLNIKFAGKEKTPEEKASVDAKFDKEAYRALAEIARLPNLTEEQRAAFIQSLKDDPSGSKAILAEAKKVNDAQAPKGSHHHHHH

SEQ ID NO: 148 - protein, 129 aa, synthetic construct
QYTGTAQHDEAQQNAFYQVLNMPNLNADQRNGFIQSLKDDPSQSANVLGEAQKLNDSQAPKASVDAKFDKEAYRALAEIARLPNLTEEQRAAFIQSLKDDPSGSKAILAEAKKVNDAQAPKGSHHHHHH

SEQ ID NO: 149 - protein, 134 aa, synthetic construct
QYTGTADAQQNKFNKDQQSAFYEILNMPNLNEEQRNGFIQSLKDDPSQSTNVLGEAKKLNESQAPKASVDAKFDKEAYRALAEIARLPNLTEEQRAAFIQSLKDDPSGSKAILAEAKKVNDAQAPKGSHHHHHH

SEQ ID NO: 150 - protein, 131 aa, synthetic construct
QYTGTADNKFNKEQQNAFYEILHLPNLTEEQRNGFIQSLKDDPSVSKEILAEAKKLNDAQAPKASVDAKFDKEAYRALAEIARLPNLTEEQRAAFIQSLKDDPSGSKAILAEAKKVNDAQAPKGSHHHHHH

SEQ ID NO: 151 - protein, 131 aa, synthetic construct
QYTGTADNKFNKEQQNAFYEILHLPNLNEEQRNGFIQSLKDDPSQSANLLAEAKKLNDAQAPKASVDAKFDKEAYRALAEIARLPNLTEEQRAAFIQSLKDDPSGSKAILAEAKKVNDAQAPKGSHHHHHH

SEQ ID NO: 152 - protein, 131 aa, synthetic construct
QYTGTADNNFNKEQQNAFYEILNMPNLNEEQRNGFIQSLKDDPSQSANLLAEAKKLNESQAPKASVDAKFDKEAYRALAEIARLPNLTEEQRAAFIQSLKDDPSGSKAILAEAKKVNDAQAPKGSHHHHHH

SEQ ID NO: 153 - protein, 260 aa, synthetic construct
EVQLLESGGGLVQPGGSLRLSCAVSGIDLSNYAINWVRQAPGKGLEWIGIIWASGTTFYATWAKGRFTISRDNSKNTVYLQMNSLRAEDTAVYYCARTVPGYSTAPYFDLWGQGTLVTVSSGGGGSGGGGSGGGGSDIQMTQSPSSVSASVGDRVTITCQSSPSVWSNFLSWYQQKPGKAPKLLIYEASKLTSGVPSRFSGSGSGTDFTLTISSLQPEDFATYYCGGGYSSISDTTFGGGTKVEIKRTVQASGSHHHHHH

SEQ ID NO: 154 - protein, 320 aa, synthetic construct
EVQLLESGGGLVQPGGSLRLSCAVSGIDLSNYAINWVRQAPGKGLEWIGIIWASGTTFYATWAKGRFTISRDNSKNTVYLQMNSLRAEDTAVYYCARTVPGYSTAPYFDLWGQGTLVTVSSGGGGSGGGGSGGGGSDIQMTQSPSSVSASVGDRVTITCQSSPSVWSNFLSWYQQKPGKAPKLLIYEASKLTSGVPSRFSGSGSGTDFTLTISSLQPEDFATYYCGGGYSSISDTTFGGGTKVEIKRTVQASVDAKFDKEAYRALAEIARLPNLTEEQRAAFIQSLKDDPSGSKAILAEAKKVNDAQAPKASGSHHHHHH

SEQ ID NO: 155 - protein, 200 aa, synthetic construct
  SIGNAL 1..4
AQGTQVQLQQSGGGSVQAGGSLRLSCTISGRTLSDYTMGWFRQRPGKEREFVAAISWSGAYTKYADSVKGRFTISRDNAKNTVYLQMNSLKPEDTAVYYCAAGPTGLLSKKATPADYDYWGQGTQVTVSSQASVDAKFDKEAYRALAEIARLPNLTEEQRAAFIQSLKDDPSGSKAILAEAKKVNDAQAPKGSHHHHHHC

SEQ ID NO: 156 - protein, 26 aa, synthetic construct
VDQLQESGGGSVQAGEALRLSCVGSG

SEQ ID NO: 157 - protein, 26 aa, Lama glama
QVQLQESGGGLVQPGGSLRLSCAASG

SEQ ID NO: 158 - protein, 26 aa, Lama glama
QVQLQESGGGLVQPGGSLRLSCAASG

SEQ ID NO: 159 - protein, 26 aa, Lama glama
QVQLQESGGGLVQPGGSLRLSCAASG

SEQ ID NO: 160 - protein, 26 aa, synthetic construct
QVQLQESGGGSVQAGGSLRLSCVASG

SEQ ID NO: 161 - protein, 26 aa, synthetic construct
QVQLQESGGGSVQAGGSLTLSCVASG

SEQ ID NO: 162 - protein, 26 aa, synthetic construct
QVQLQESGGGSVQAGGSLRLSCTASG

SEQ ID NO: 163 - protein, 26 aa, synthetic construct
QVQLQESGGGSVQAGGSLTLSCTASG

SEQ ID NO: 164 - protein, 26 aa, synthetic construct
QVQLQQSGGGSVQAGGSLRLSCTISG

SEQ ID NO: 165 - protein, 26 aa, synthetic construct
QVQLQESGGGSVQAGGSLRLSCTISG

SEQ ID NO: 166 - protein, 26 aa, synthetic construct
QVQLQQSGGGSVQAGGSLRLSCTVSG

SEQ ID NO: 167 - protein, 26 aa, synthetic construct
QVQLQQSGGGSVQAGGSLTLSCTISG

SEQ ID NO: 168 - protein, 26 aa, synthetic construct
QVQLVQSGGGSVQAGGSLRLSCTISG

SEQ ID NO: 169 - protein, 26 aa, synthetic construct
QVQLEQSGGGSVQAGGSLRLSCTISG

SEQ ID NO: 170 - protein, 26 aa, synthetic construct
QVQLQQSGGGSVQSGGSLRLSCTISG

SEQ ID NO: 171 - protein, 26 aa, synthetic construct
QVQLQQSGGGSVQTGGSLRLSCTISG

SEQ ID NO: 172 - protein, 26 aa, synthetic construct
QVQLQQSGGGSVQAGGSLKLSCTISG

SEQ ID NO: 173 - protein, 26 aa, synthetic construct
QVQLQQSGGGSVQAGGSLSLSCTISG

SEQ ID NO: 174 - protein, 26 aa, synthetic construct
QVQLQQSGGGSVQAGGSLRLSCVISG

SEQ ID NO: 175 - protein, 26 aa, synthetic construct
QVQLQQSGGGSVQAGGSLRLSCSISG

SEQ ID NO: 176 - protein, 26 aa, synthetic construct
QVQLQQSGGGSVQAGGSLRLSCAISG

SEQ ID NO: 177 - protein, 26 aa, synthetic construct
QVQLQQSGGGSVQAGGSLRLSCTSSG

SEQ ID NO: 178 - protein, 14 aa, Camelus dromedarius
WFRQAPGKEREGVA

SEQ ID NO: 179 - protein, 14 aa, Lama glama
WFRQAPGKQREFVA

SEQ ID NO: 180 - protein, 14 aa, Lama glama
WFRQAPGKQREFVA

SEQ ID NO: 181 - protein, 14 aa, Lama glama
WFRQAPGKQREFVA

SEQ ID NO: 182 - protein, 14 aa, synthetic construct
WFRQPPGKAREFVA

SEQ ID NO: 183 - protein, 14 aa, synthetic construct
WFRQRPGKAREFVA

SEQ ID NO: 184 - protein, 14 aa, synthetic construct
WFRQRPGKAREGVA

SEQ ID NO: 185 - protein, 14 aa, synthetic construct
WFRQRPGKEREFVA

SEQ ID NO: 186 - protein, 14 aa, synthetic construct
WFRQPPGKEREFVA

SEQ ID NO: 187 - protein, 14 aa, synthetic construct
WFRQTPGKEREFVA

SEQ ID NO: 188 - protein, 14 aa, synthetic construct
WFRQIPGKEREFVA

SEQ ID NO: 189 - protein, 14 aa, synthetic construct
WFRQKPGKEREFVA

SEQ ID NO: 190 - protein, 14 aa, synthetic construct
WFRQAPGKEREFVA

SEQ ID NO: 191 - protein, 14 aa, synthetic construct
WFRQRPGGEREFVA

SEQ ID NO: 192 - protein, 14 aa, synthetic construct
WFRQRPGQEREFVA

SEQ ID NO: 193 - protein, 14 aa, synthetic construct
WFRQRPGREREFVA

SEQ ID NO: 194 - protein, 14 aa, synthetic construct
WFRQRPGKQREFVA

SEQ ID NO: 195 - protein, 14 aa, synthetic construct
WFRQRPGKDREFVA

SEQ ID NO: 196 - protein, 14 aa, synthetic construct
WFRQRPGKGREFVA

SEQ ID NO: 197 - protein, 14 aa, synthetic construct
WFRQRPGKELEFVA

SEQ ID NO: 198 - protein, 14 aa, synthetic construct
WFRQRPGKEIEFVA

SEQ ID NO: 199 - protein, 14 aa, synthetic construct
WFRQRPGKERELVA

SEQ ID NO: 200 - protein, 14 aa, synthetic construct
WFRQRPGKEREYVA

SEQ ID NO: 201 - protein, 14 aa, synthetic construct
WFRQRPGKERESVA

SEQ ID NO: 202 - protein, 14 aa, synthetic construct
WFRQRPGKERETVA

SEQ ID NO: 203 - protein, 39 aa, Camelus dromedarius
YADSVKGRFTITRDNVKNTMYLQMPSLKPEDSAKYYCAA

SEQ ID NO: 204 - protein, 39 aa, Lama glama
YTDSVKGRFTISRDNAKTTVYLQMNSLKPEDTAVYYCAA

SEQ ID NO: 205 - protein, 39 aa, Lama glama; identical to SEQ ID NO: 204

SEQ ID NO: 206 - protein, 39 aa, Lama glama; identical to SEQ ID NO: 204

SEQ ID NO: 207 - protein, 39 aa, synthetic construct
YADSVKGRFTISRDNAKNTVYLQMNSLKPEDTAVYYCAA

SEQ ID NO: 208 - protein, 39 aa, synthetic construct
YNDSVKGRFTISRDNAKNTVYLQMNSLKPEDTAVYYCAA

SEQ ID NO: 209 - protein, 39 aa, synthetic construct
YQDSVKGRFTISRDNAKNTVYLQMNSLKPEDTAVYYCAA

SEQ ID NO: 210 - protein, 39 aa, synthetic construct
YTDSVKGRFTISRDNAKNTVYLQMNSLKPEDTAVYYCAA

SEQ ID NO: 211 - protein, 39 aa, synthetic construct
YSDSVKGRFTISRDNAKNTVYLQMNSLKPEDTAVYYCAA

SEQ ID NO: 212 - protein, 39 aa, synthetic construct
YVDSVKGRFTISRDNAKNTVYLQMNSLKPEDTAVYYCAA

SEQ ID NO: 213 - protein, 39 aa, synthetic construct
YADSVKGRFTISRDNAKTTVYLQMNSLKPEDTAVYYCAA

SEQ ID NO: 214 - protein, 39 aa, synthetic construct
YADSVKGRFTISRDNAKSTVYLQMNSLKPEDTAVYYCAA

SEQ ID NO: 215 - protein, 39 aa, synthetic construct
YADSVKGRFTISRDNAKETVYLQMNSLKPEDTAVYYCAA

SEQ ID NO: 216 - protein, 39 aa, synthetic construct
YADSVKGRFTISRDNAKQTVYLQMNSLKPEDTAVYYCAA

SEQ ID NO: 217 - protein, 39 aa, synthetic construct
YADSVKGRFTISRDNAKDTVYLQMNSLKPEDTAVYYCAA

SEQ ID NO: 218 - protein, 39 aa, synthetic construct
YADSVKGRFTISRDNAKNTVLLQMNSLKPEDTAVYYCAA

SEQ ID NO: 219 - protein, 39 aa, synthetic construct
YADSVKGRFTISRDNAKNTVVLQMNSLKPEDTAVYYCAA

SEQ ID NO: 220 - protein, 39 aa, synthetic construct
YADSVKGRFTISRDNAKNTVALQMNSLKPEDTAVYYCAA

SEQ ID NO: 221 - protein, 39 aa, synthetic construct
YADSVKGRFTISRDNAKNTVFLQMNSLKPEDTAVYYCAA

SEQ ID NO: 222 - protein, 39 aa, synthetic construct
YADSVKGRFTISRDNAKNTVWLQMNSLKPEDTAVYYCAA

SEQ ID NO: 223 - protein, 39 aa, synthetic construct
YADSVKGRFTISRDNAKNTVYLQMNNLKPEDTAVYYCAA

SEQ ID NO: 224 - protein, 39 aa, synthetic construct
YADSVKGRFTISRDNAKNTVYLQMNTLKPEDTAVYYCAA

SEQ ID NO: 225 - protein, 39 aa, synthetic construct
YADSVKGRFTISRDNAKNTVYLQMNQLKPEDTAVYYCAA

SEQ ID NO: 226 - protein, 39 aa, synthetic construct
YADSVKGRFTISRDNAKNTVYLQMNSLKPEDTADYYCAA

SEQ ID NO: 227 - protein, 39 aa, synthetic construct
YADSVKGRFTISRDNAKNTVYLQMNSLKPEDTAAYYCAA

SEQ ID NO: 228 - protein, 39 aa, synthetic construct
YADSVKGRFTISRDNAKNTVYLQMNSLKPEDTAEYYCAA

SEQ ID NO: 229 - protein, 39 aa, synthetic construct
YADSVKGRFTISRDNAKNTVYLQMNSLKPEDTAIYYCAA

SEQ ID NO: 230 - protein, 39 aa, synthetic construct
YADSVKGRFTISRDNAKNTVYLQMNSLKPEDTALYYCAA

SEQ ID NO: 231 - protein, 11 aa, Lama glama
WGQGTQVTVSS

SEQ ID NO: 232 - protein, 76 aa, synthetic construct
AQYEDGKQYTGTAQHDEAQQNAFYQVLNMPNLNADQRNGFIQSLKDDPSQSANVLGEAQKLNDSQAPKASHHHHHH

SEQ ID NO: 233 - protein, 81 aa, synthetic construct
AQYEDGKQYTGTADAQQNKFNKDQQSAFYEILNMPNLNEEQRNGFIQSLKDDPSQSTNVLGEAKKLNESQAPKASHHHHHH

SEQ ID NO: 234 - protein, 78 aa, synthetic construct
AQYEDGKQYTGTADNNFNKEQQNAFYEILNMPNLNEEQRNGFIQSLKDDPSQSANLLAEAKKLNESQAPKASHHHHHH

SEQ ID NO: 235 - protein, 58 aa, synthetic construct
  VARIANT 9: note = X is L or E or R or A or Y
  VARIANT 10: note = X is L or E or R or A or Y
  VARIANT 11: note = X is L or E or R or A or Y
  VARIANT 13: note = X is L or E or R or A or Q
  VARIANT 14: note = X is L or E or R or A or Q or K
  VARIANT 17: note = X is L or E or R or A
  VARIANT 18: note = X is L or E or R or A
  VARIANT 28: note = X is L or E or R or A
  VARIANT 29: note = X is L or E or R or A
  VARIANT 33: note = X is T or S or G or Q or A or E or H or R
  VARIANT 40: note = X is E or G or R or D or K or Q or H or S
  VARIANT 51: note = X is L or V or S or I or R or G
VDAKFDKEXXXAXXEIXXLPNLTEEQRXXFIQXLKDDPSXSKAILAEAKKXNDAQAPK